European Patent Application EP 4 759 825 A1, published June 17, 2026. Title: peptide fragment and use thereof. Applicant: TOAGOSEI CO., LTD. Application JP. The sequence listing filed with the application follows.

SEQUENCE LISTING (9 sequences)

SEQ ID NO: 1 - protein, 18 aa, synthetic construct
YLIQFKKRTLRKSNRKKR

SEQ ID NO: 2 - protein, 18 aa, synthetic construct
FQILYKKRTLRKSNRKKR

SEQ ID NO: 3 - protein, 18 aa, synthetic construct
YQFLIKKRTLRKSNRKKR

SEQ ID NO: 4 - protein, 18 aa, synthetic construct
ILFQYKKRTLRKSNRKKR

SEQ ID NO: 5 - protein, 13 aa, synthetic construct
KKRTLRKSNRKKR

SEQ ID NO: 6 - protein, 5 aa, synthetic construct
YLIQF

SEQ ID NO: 7 - protein, 5 aa, synthetic construct
FQILY

SEQ ID NO: 8 - protein, 5 aa, synthetic construct
YQFLI

SEQ ID NO: 9 - protein, 5 aa, synthetic construct
ILFQY